European Patent Application EP 4 471 055 A1, published December 4, 2024. Title: EPITOPE PEPTIDE AND ANTIBODY FOR TREATING HBV INFECTION AND RELATED DISEASES. Applicant: XIAMEN UNIVERSITY. Application CN PCT/CN2023/073343, filed January 20, 2023. The sequence listing filed with the application follows.

SEQUENCE LISTING (51 sequences)

SEQ ID NO: 1 - protein, 8 aa, synthetic construct
  source 1..8: note = 125s VHH-CDR1
GGTISAYA

SEQ ID NO: 2 - protein, 8 aa, synthetic construct
  source 1..8: note = 125s VHH-CDR2
ISWTTSSA

SEQ ID NO: 3 - protein, 12 aa, synthetic construct
  source 1..12: note = 125s VHH-CDR3
NDRVSDTVGFGS

SEQ ID NO: 4 - protein, 25 aa, synthetic construct
  source 1..25: note = 125s VHH-FR1
QLQLVESGGGLVQAGGSLRLSCAAS

SEQ ID NO: 5 - protein, 17 aa, synthetic construct
  source 1..17: note = 125s VHH-FR2
MGWFRQAPGKDREFVAG

SEQ ID NO: 6 - protein, 38 aa, synthetic construct
  source 1..38: note = 125s VHH-FR3
YYTDSVKGRFTISRDFAKNTVYLQMNSLKPEDTAVYYC

SEQ ID NO: 7 - protein, 11 aa, synthetic construct
  source 1..11: note = 125s VHH-FR4
WGQGTQVTVSS

SEQ ID NO: 8 - protein, 119 aa, synthetic construct
  source 1..119: note = 125s VHH
QLQLVESGGGLVQAGGSLRLSCAASGGTISAYAMGWFRQAPGKDREFVAGISWTTSSAYYTDSVKGRFTISRDFAKNTVYLQMNSLKPEDTAVYYCNDRVSDTVGFGSWGQGTQVTVSS

SEQ ID NO: 9 - protein, 25 aa, synthetic construct [sequence omitted]

SEQ ID NO: 10 - protein, 17 aa, synthetic construct
  source 1..17: note = h125s-26 VHH-FR2
MGWFRQAPGKDREFVAG

SEQ ID NO: 11 - protein, 38 aa, synthetic construct; identical to SEQ ID NO: 6
  source 1..38: note = h125s-26 VHH-FR3

SEQ ID NO: 12 - protein, 11 aa, synthetic construct
  source 1..11: note = h125s-26 VHH-FR4
WGQGTLVTVSS

SEQ ID NO: 13 - protein, 119 aa, synthetic construct
  source 1..119: note = h125s-26 VHH
EVQLVESGGGLVQPGGSLRLSCAASGGTISAYAMGWFRQAPGKDREFVAGISWTTSSAYYTDSVKGRFTISRDFAKNTVYLQMNSLKPEDTAVYYCNDRVSDTVGFGSWGQGTLVTVSS

SEQ ID NO: 14 - protein, 231 aa, synthetic construct
  source 1..231: note = hIgG1-Fc
PKSCDKTHTCPPCPAPELLGGPSVFLFPPKPKDTLMISRTPEVTCVVVDVSHEDPEVKFNWYVDGVEVHNAKTKPREEQYNSTYRVVSVLTVLHQDWLNGKEYKCKVSNKALPAPIEKTISKAKGQPREPQVYTLPPSRDELTKNQVSLTCLVKGFYPSDIAVEWESNGQPENNYKTTPPVLDSDGSFFLYSKLTVDKSRWQQGNVFSCSVMHEALHNHYTQKSLSLSPGK

SEQ ID NO: 15 - protein, 237 aa, synthetic construct
  source 1..237: note = mIgG2-Fc
PRVPITQNPCPPLKECPPCAAPDLLGGPSVFIFPPKIKDVLMISLSPMVTCVVVDVSEDDPDVQISWFVNNVEVHTAQTQTHREDYNSTLRVVSALPIQHQDWMSGKEFKCKVNNRALPSPIEKTISKPRGPVRAPQVYVLPPPAEEMTKKEFSLTCMITGFLPAEIAVDWTSNGRTEQNYKNTATVLDSDGSYFMYSKLRVQKSTWERGSLFACSVVHEGLHNHLTTKTISRSLGK

SEQ ID NO: 16 - protein, 74 aa, synthetic construct
  source 1..74: note = HBsAg extracellular segment S1
QGMLPVCPLIPGSSTTSTGPCKTCTTPAQGNSTFPSCCCIKPTDGNCTCIPIPSSWAFAKYLWEWASVRFSWLS

SEQ ID NO: 17 - protein, 56 aa, synthetic construct
  source 1..56: note = HBsAg extracellular segment S2
QGMLPVCPLIPGSSTTSTGPCKTCTTPAQGNSTFPSCCCIKPTDGNCTCIPIPSSW

SEQ ID NO: 18 - protein, 39 aa, synthetic construct
  source 1..39: note = HBsAg extracellular segment S3
TGPCKTCTTPAQGNSTFPSCCCIKPTDGNCTCIPIPSSW

SEQ ID NO: 19 - protein, 18 aa, synthetic construct
  source 1..18: note = HBsAg extracellular segment S4
AFAKYLWEWASVRFSWLS

SEQ ID NO: 20 - protein, 36 aa, synthetic construct
  source 1..36: note = HBsAg extracellular segment S5
CIKPTDGNCTCIPIPSSWAFAKYLWEWASVRFSWLS

SEQ ID NO: 21 - protein, 57 aa, synthetic construct
  source 1..57: note = HBsAg extracellular segment S6
TGPCKTCTTPAQGNSTFPSCCCIKPTDGNCTCIPIPSSWAFAKYLWEWASVRFSWLS

SEQ ID NO: 22 - protein, 74 aa, synthetic construct
  source 1..74: note = HBsAg extracellular segment S1- F158A
QGMLPVCPLIPGSSTTSTGPCKTCTTPAQGNSTFPSCCCIKPTDGNCTCIPIPSSWAAAKYLWEWASVRFSWLS

SEQ ID NO: 23 - protein, 74 aa, synthetic construct
  source 1..74: note = HBsAg extracellular segment S1- K160A
QGMLPVCPLIPGSSTTSTGPCKTCTTPAQGNSTFPSCCCIKPTDGNCTCIPIPSSWAFAAYLWEWASVRFSWLS

SEQ ID NO: 24 - protein, 74 aa, synthetic construct
  source 1..74: note = HBsAg extracellular segment S1- Y161A
QGMLPVCPLIPGSSTTSTGPCKTCTTPAQGNSTFPSCCCIKPTDGNCTCIPIPSSWAFAKALWEWASVRFSWLS

SEQ ID NO: 25 - protein, 74 aa, synthetic construct
  source 1..74: note = HBsAg extracellular segment S1- L162A
QGMLPVCPLIPGSSTTSTGPCKTCTTPAQGNSTFPSCCCIKPTDGNCTCIPIPSSWAFAKYAWEWASVRFSWLS

SEQ ID NO: 26 - protein, 74 aa, synthetic construct
  source 1..74: note = HBsAg extracellular segment S1- W163A
QGMLPVCPLIPGSSTTSTGPCKTCTTPAQGNSTFPSCCCIKPTDGNCTCIPIPSSWAFAKYLAEWASVRFSWLS

SEQ ID NO: 27 - protein, 74 aa, synthetic construct
  source 1..74: note = HBsAg extracellular segment S1- W165A
QGMLPVCPLIPGSSTTSTGPCKTCTTPAQGNSTFPSCCCIKPTDGNCTCIPIPSSWAFAKYLWEAASVRFSWLS

SEQ ID NO: 28 - protein, 74 aa, synthetic construct
  source 1..74: note = HBsAg extracellular segment S1- S167A
QGMLPVCPLIPGSSTTSTGPCKTCTTPAQGNSTFPSCCCIKPTDGNCTCIPIPSSWAFAKYLWEWAAVRFSWLS

SEQ ID NO: 29 - protein, 74 aa, synthetic construct
  source 1..74: note = HBsAg extracellular segment S1- V168A
QGMLPVCPLIPGSSTTSTGPCKTCTTPAQGNSTFPSCCCIKPTDGNCTCIPIPSSWAFAKYLWEWASARFSWLS

SEQ ID NO: 30 - protein, 74 aa, synthetic construct
  source 1..74: note = HBsAg extracellular segment S1- R169A
QGMLPVCPLIPGSSTTSTGPCKTCTTPAQGNSTFPSCCCIKPTDGNCTCIPIPSSWAFAKYLWEWASVAFSWLS

SEQ ID NO: 31 - protein, 74 aa, synthetic construct
  source 1..74: note = HBsAg extracellular segment S1- F170A
QGMLPVCPLIPGSSTTSTGPCKTCTTPAQGNSTFPSCCCIKPTDGNCTCIPIPSSWAFAKYLWEWASVRASWLS

SEQ ID NO: 32 - protein, 74 aa, synthetic construct
  source 1..74: note = HBsAg extracellular segment S1- S171A
QGMLPVCPLIPGSSTTSTGPCKTCTTPAQGNSTFPSCCCIKPTDGNCTCIPIPSSWAFAKYLWEWASVRFAWLS

SEQ ID NO: 33 - protein, 74 aa, synthetic construct
  source 1..74: note = HBsAg extracellular segment S1- W172A
QGMLPVCPLIPGSSTTSTGPCKTCTTPAQGNSTFPSCCCIKPTDGNCTCIPIPSSWAFAKYLWEWASVRFSALS

SEQ ID NO: 34 - protein, 74 aa, synthetic construct
  source 1..74: note = HBsAg extracellular segment S1- L173A
QGMLPVCPLIPGSSTTSTGPCKTCTTPAQGNSTFPSCCCIKPTDGNCTCIPIPSSWAFAKYLWEWASVRFSWAS

SEQ ID NO: 35 - protein, 74 aa, synthetic construct
  source 1..74: note = HBsAg extracellular segment S1- S174A
QGMLPVCPLIPGSSTTSTGPCKTCTTPAQGNSTFPSCCCIKPTDGNCTCIPIPSSWAFAKYLWEWASVRFSWLA

SEQ ID NO: 36 - protein, 226 aa, synthetic construct
  source 1..226: note = HBsAg
MENIASGLLGPLLVLQAGFFLLTKILTIPKSLDSWWTSLNFLGGTPVCLGQNSQSQISNHSPTCCPPICPGYRWMCLRRFIIFLCILLLCLIFLLVLLDYQGMLPVCPLIPGSSTTSTGPCKTCTTPAQGNSTFPSCCCIKPTDGNCTCIPIPSSWAFAKYLWEWASVRFSWLSLLVPFVQWFVGLSPTVWLSVIWMMWYWGPSLYNILSPFMPLLPIFCCLWVYS

SEQ ID NO: 37 - protein, 4 aa, synthetic construct
  source 1..4: note = HBsAg aa163-166
WEWA

SEQ ID NO: 38 - protein, 18 aa, synthetic construct
  source 1..18: note = HBsAg aa157-174 (genotype C)
AFARFLWEWASVRFSWLS

SEQ ID NO: 39 - protein, 18 aa, synthetic construct
  source 1..18: note = HBsAg aa157-174 (genotype D/E)
AFGKFLWEWASARFSWLS

SEQ ID NO: 40 - protein, 18 aa, synthetic construct
  source 1..18: note = HBsAg aa157-174 (genotype F)
ALGKYLWEWASARFSWLS

SEQ ID NO: 41 - protein, 18 aa, synthetic construct
  source 1..18: note = HBsAg aa157-174 (genotype G)
AFAKYLWEWASVHFSWLS

SEQ ID NO: 42 - protein, 18 aa, synthetic construct
  source 1..18: note = HBsAg aa157-174 (genotype H)
AFGKYLWEWASARFSWLS

SEQ ID NO: 43 - protein, 18 aa, synthetic construct
  source 1..18: note = HBsAg aa157-174 (genotype I)
AFAKYLWEWASARFSWLS

SEQ ID NO: 44 - protein, 18 aa, synthetic construct
  source 1..18: note = HBsAg aa157-174 (genotype J)
AFAKFLWEWASVRFSWLS

SEQ ID NO: 45 - protein, 182 aa, synthetic construct
  source 1..182: note = Murine ferritin
MTTASPSQVRQNYHQDAEAAINRQINLELYASYVYLSMSCYFDRDDVALKNFAKYFLHQSHEEREHAEKLMKLQNQRGGRIFLQDIKKPDRDDWESGLNAMECALHLEKSVNQSLLELHKLATDKNDPHLCDFIETYYLSEQVKSIKELGDHVTNLRKMGAPEAGMAEYLFDKHTLGHGDES

SEQ ID NO: 46 - protein, 16 aa, synthetic construct
  source 1..16: note = SpyTag
AHIVMVDAYKPTKSYY

SEQ ID NO: 47 - protein, 139 aa, synthetic construct
  source 1..139: note = SpyCatcher full-length sequence
MSYYHHHHHHDYDIPTTENLYFQGAMVDTLSGLSSEQGQSGDMTIEEDSATHIKFSKRDEDGKELAGATMELRDSSGKTISTWISDGQVKDFYLYPGKYTFVETAAPDGYEVATAITFTVNEQGQVTVNGKATKGDAHI

SEQ ID NO: 48 - protein, 116 aa, synthetic construct
  source 1..116: note = SpyCatcher truncated sequence
MSYYHHHHHHDYDIPTTENLYFQGDSATHIKFSKRDEDGKELAGATMELRDSSGKTISTWISDGQVKDFYLYPGKYTFVETAAPDGYEVATAITFTVNEQGQVTVNGKATKGDAHI

SEQ ID NO: 49 - protein, 213 aa, synthetic construct
  source 1..213: note = SpyTag-murine ferritin
AHIVMVDAYKPTKSYYGGGGSGGGGSGGGGSMTTASPSQVRQNYHQDAEAAINRQINLELYASYVYLSMSCYFDRDDVALKNFAKYFLHQSHEEREHAEKLMKLQNQRGGRIFLQDIKKPDRDDWESGLNAMECALHLEKSVNQSLLELHKLATDKNDPHLCDFIETYYLSEQVKSIKELGDHVTNLRKMGAPEAGMAEYLFDKHTLGHGDES

SEQ ID NO: 50 - protein, 149 aa, synthetic construct
  source 1..149: note = SpyCatcher-Cter
MSYYHHHHHHDYDIPTTENLYFQGDSATHIKFSKRDEDGKELAGATMELRDSSGKTISTWISDGQVKDFYLYPGKYTFVETAAPDGYEVATAITFTVNEQGQVTVNGKATKGDAHIGGGGSGGGGSGGGGSAFAKYLWEWASVRFSWLS

SEQ ID NO: 51 - protein, 18 aa, synthetic construct
  source 1..18: note = General formula of aa157-174
  VARIANT 2: note = X is F or L
  VARIANT 3: note = X is A or G
  VARIANT 4: note = X is K or R
  VARIANT 5: note = X is any natural amino acid
  VARIANT 6: note = X is any natural amino acid
  VARIANT 11: note = X is any natural amino acid
  VARIANT 12: note = X is any natural amino acid
  VARIANT 13: note = X is any natural amino acid
  VARIANT 14: note = X is any natural amino acid
  VARIANT 16: note = X is any natural amino acid
  VARIANT 17: note = X is any natural amino acid
  VARIANT 18: note = X is any natural amino acid
AXXXXXWEWAXXXXSXXX